European Patent Specification EP 3 810 167 B1, published December 11, 2024. Title: BICYCLIC PEPTIDE LIGANDS SPECIFIC FOR NECTIN-4. Applicant: BicycleTx Limited. The sequence listing filed with the application follows.

SEQUENCE LISTING (2 sequences)

SEQ ID NO: 1 - protein, 15 aa, Artificial Sequence
  synthetic
  Xaa (3)..(3): 1-Nal
  Xaa (4)..(4): dD
  Xaa (7)..(7): HArg
  Xaa (13)..(13): HyP
CPXXCMXDWSTPXWC

SEQ ID NO: 2 - protein, 18 aa, Artificial Sequence
  synthetic
  Xaa (18)..(18): Sar6-K(Fl)
ACPFGCHTDWSWPIWCAX